European Patent Application EP 4 257 153 A1, published October 11, 2023. Title: ANTIBODY-DRUG CONJUGATE, AND INTERMEDIATE THEREOF, PREPARATION METHOD THEREFOR, AND APPLICATION THEREOF. Applicant: SHANGHAI FUDAN-ZHANGJIANG BIO-PHARMACEUTICAL CO., LTD. The sequence listing filed with the application follows.

SEQUENCE LISTING (4 sequences)

SEQ ID NO: 1 - protein, 220 aa, Homo sapiens
DIEMTQSPDSLAVSLGERATINCRSSQSVLYSSSNRNYLAWYQQNPGQPPKLLIYWASTRESGVPDRFSGSGSGTDFTLTISSLQAEDVAVYYCQQYYSTPRTFGQGTKVEIKRTVAAPSVFIFPPSDEQLKSGTASVVCLLNNFYPREAKVQWKVDNALQSGNSQESVTEQDSKDSTYSLSSTLTLSKADYEKHKVYACEVTHQGLSSPVTKSFNRGEC

SEQ ID NO: 2 - protein, 447 aa, Homo sapiens
QVQLQQWGAGLLKPSETLSLTCAVYGGSFSGYYWSWIRQPPGKGLEWIGEINHSGSTNYNPSLKSRVTISVETSKNQFSLKLSSVTAADTAVYYCARDKWTWYFDLWGRGTLVTVSSASTKGPSVFPLAPSSKSTSGGTAALGCLVKDYFPEPVTVSWNSGALTSGVHTFPAVLQSSGLYSLSSVVTVPSSSLGTQTYICNVNHKPSNTKVDKRVEPKSCDKTHTCPPCPAPELLGGPSVFLFPPKPKDTLMISRTPEVTCVVVDVSHEDPEVKFNWYVDGVEVHNAKTKPREEQYNSTYRVVSVLTVLHQDWLNGKEYKCKVSNKALPAPIEKTISKAKGQPREPQVYTLPPSREEMTKNQVSLTCLVKGFYPSDIAVEWESNGQPENNYKTTPPVLDSDGSFFLYSKLTVDKSRWQQGNVFSCSVMHEALHNHYTQKSLSLSPGK

SEQ ID NO: 3 - protein, 447 aa, Artificial Sequence
  FDA028 heavy chain
QVQLQQWGAGLLKPSETLSLTCAVYGGSFSGYYWSWIRQPPGKGLEWIGEINHSGSTNYNPSLKSRVTISVETSKNQFSLKLSSVTAADTAVYYCARDKWTWYFDLWGRGTLVTVSSASTKGPSVFPLAPSSKSTSGGTAALGCLVKDYFPEPVTVSWNSGALTSGVHTFPAVLQSSGLYSLSSVVTVPSSSLGTQTYICNVNHKPSNTKVDKKVEPKSCDKTHTCPPCPAPPVAGGPSVFLFPPKPKDTLMISRTPEVTCVVVDVSHEDPEVKFNWYVDGVEVHNAKTKPREEQYNSTYRVVSVLTVLHQDWLNGKEYKCKVSNKALPAPIEKTISKAKGQPREPQVYTLPPSREEMTKNQVSLTCLVKGFYPSDIAVEWESNGQPENNYKTTPPVLDSDGSFFLYSKLTVDKSRWQQGNVFSCSVMHEALHNHYTQKSLSLSPGK

SEQ ID NO: 4 - protein, 447 aa, Artificial Sequence
  FDA029 heavy chain
QVQLQQWGAGLLKPSETLSLTCAVYGGSFSGYYWSWIRQPPGKGLEWIGEINHSGSTNYNPSLKSRVTISVETSKNQFSLKLSSVTAADTAVYYCARDKWTWYFDLWGRGTLVTVSSASTKGPSVFPLAPSSKSTSGGTAALGCLVKDYFPEPVTVSWNSGALTSGVHTFPAVLQSSGLYSLSSVVTVPSSSLGTQTYICNVNHKPSNTKVDKKVEPKSCDKTHTCPPCPAPEFEGGPSVFLFPPKPKDTLMISRTPEVTCVVVDVSHEDPEVKFNWYVDGVEVHNAKTKPREEQYNSTYRVVSVLTVLHQDWLNGKEYKCKVSNKALPASIEKTISKAKGQPREPQVYTLPPSREEMTKNQVSLTCLVKGFYPSDIAVEWESNGQPENNYKTTPPVLDSDGSFFLYSKLTVDKSRWQQGNVFSCSVMHEALHNHYTQKSLSLSPGK